European Patent Application EP 4 403 624 A1, published July 24, 2024. Title: Scalp microbiome complex and its use for improving hair or scalp condition. Applicant: Cosmax, INC. Application KR 10-2021-0122765, filed September 14, 2021. The sequence listing filed with the application follows.

SEQUENCE LISTING (8 sequences)

SEQ ID NO: 1 - DNA, 1363 bp, synthetic construct
  source 1..1363: mol_type = other DNA
ctggctcagaacgaacgctggcggcaggcctaacacatgcaagtcgagcgaacccttcggggttagcggcggacgggtgagtaacgcgtgggaatatgccctttgctacggaatagccccgggaaactgggagtaataccgtatacgccctttgggggaaagatttatcggcaaaggattagcccgcgttggattaggtagttggtggggtaatggcctaccaagccgacgatccatagctggtttgagaggatgatcagccacactgggactgagacacggcccagactcctacgggaggcagcagtggggaatcttagacaatgggggcaaccctgatctagccatgccgcgtgagtgatgaaggccctagggttgtaaagctctttcagctgggaagataatgacggtaccagcagaagaagccccggctaactccgtgccagcagccgcggtaatacggagggggctagcgttgttcggaattactgggcgtaaagcgcacgtaggcggaccggaaagttgggggtgaaatcccggggctcaacctcggaactgccttcaaaactatcggtctggagttcgagagaggtgagtggaattccgagtgtagaggtgaaattcgtagatattcggaggaacaccagtggcgaaggcggctcactggctcgatactgacgctgaggtgcgaaagcgtggggagcaaacaggattagataccctggtagtccacgccgtaaacgatgaatgccagtcgtcgggcagcatgctgttcggtgacacacctaacggattaagcattccgcctggggagtacggtcgcaagattaaaactcaaaggaattgacgggggcccgcacaagcggtggagcatgtggtttaattcgaagcaacgcgcagaaccttaccaacccttgacatcgcaggaccgctccagagatggagttttctcgtaagagacctgtggacaggtgctgcatggctgtcgtcagctcgtgtcgtgagatgttcggttaagtccggcaacgagcgcaacccacactcttagttgccagcatttggttgggcactctaagagaactgccgatgataagtcggaggaaggtgtggatgacgtcaagtcctcatggcccttacgggttgggctacacacgtgctacaatggtggtgacagtgggttaatccccaaaagccatctcagttcggattggggtctgcaactcgaccccatgaagttggaatcgctagtaatcgcggaacagcatgccgcggtgaatacgttcccgggccttgtacacaccgcccgtcacaccatgggagttgggtctacccgacggccgtgcgctaaccagcaatggaggca

SEQ ID NO: 2 - DNA, 1444 bp, synthetic construct
  source 1..1444: mol_type = other DNA
ctggctcaggatgaacgctggcggcgtgcctaatacatgcaagtcgagcgaacagacgaggagcttgctcctctgacgttagcggcggacgggtgagtaacacgtggataacctacctataagactgggataacttcgggaaaccggagctaataccggataatatattgaaccgcatggttcaatagtgaaagacggttttgctgtcacttatagatggatccgcgccgcattagctagttggtaaggtaacggcttaccaaggcaacgatgcgtagccgacctgagagggtgatcggccacactggaactgagacacggtccagactcctacgggaggcagcagtagggaatcttccgcaatgggcgaaagcctgacggagcaacgccgcgtgagtgatgaaggtcttcggatcgtaaaactctgttattagggaagaacaaatgtgtaagtaactatgcacgtcttgacggtacctaatcagaaagccacggctaactacgtgccagcagccgcggtaatacgtaggtggcaagcgttatccggaattattgggcgtaaagcgcgcgtaggcggttttttaagtctgatgtgaaagcccacggctcaaccgtggagggtcattggaaactggaaaacttgagtgcagaagaggaaagtggaattccatgtgtagcggtgaaatgcgcagagatatggaggaacaccagtggcgaaggcgactttctggtctgtaactgacgctgatgtgcgaaagcgtggggatcaaacaggattagataccctggtagtccacgccgtaaacgatgagtgctaagtgttagggggtttccgccccttagtgctgcagctaacgcattaagcactccgcctggggagtacgaccgcaaggttgaaactcaaaggaattgacggggacccgcacaagcggtggagcatgtggtttaattcgaagcaacgcgaagaaccttaccaaatcttgacatcctctgacccctctagagatagagttttccccttcgggggacagagtgacaggtggtgcatggttgtcgtcagctcgtgtcgtgagatgttgggttaagtcccgcaacgagcgcaacccttaagcttagttgccatcattaagttgggcactctaagttgactgccggtgacaaaccggaggaaggtggggatgacgtcaaatcatcatgccccttatgatttgggctacacacgtgctacaatggacaatacaaagggcagcgaaaccgcgaggtcaagcaaatcccataaagttgttctcagttcggattgtagtctgcaactcgactatatgaagctggaatcgctagtaatcgtagatcagcatgctacggtgaatacgttcccgggtcttgtacacaccgcccgtcacaccacgagagtttgtaacacccgaagccggtggagtaaccattg

SEQ ID NO: 3 - DNA, 21 bp, synthetic construct
  source 1..21: mol_type = other DNA
gtgcccactgaggagttcaac

SEQ ID NO: 4 - DNA, 20 bp, synthetic construct
  source 1..20: mol_type = other DNA
ccctatgtgctggccttgat

SEQ ID NO: 5 - DNA, 21 bp, synthetic construct
  source 1..21: mol_type = other DNA
tcctgccaactttgctctaca

SEQ ID NO: 6 - DNA, 21 bp, synthetic construct
  source 1..21: mol_type = other DNA
cagggctggaacagttcacat

SEQ ID NO: 7 - DNA, 20 bp, synthetic construct
  source 1..20: mol_type = other DNA
ggccatctcttgctcgaagt

SEQ ID NO: 8 - DNA, 20 bp, synthetic construct
  source 1..20: mol_type = other DNA
gagaccttcaacaccccagc